European Patent Application EP 4 261 221 A1, published October 18, 2023. Title: TARGET ANTIGEN ASSAY. Applicant: Denka Company Limited. The sequence listing filed with the application follows.

SEQUENCE LISTING (52 sequences)

SEQ ID NO: 1 - protein, 330 aa, Homo sapiens [sequence omitted]

SEQ ID NO: 2 - protein, 326 aa, Homo sapiens
ASTKGPSVFPLAPCSRSTSESTAALGCLVKDYFPEPVTVSWNSGALTSGVHTFPAVLQSSGLYSLSSVVTVPSSNFGTQTYTCNVDHKPSNTKVDKTVERKCCVECPPCPAPPVAGPSVFLFPPKPKDTLMISRTPEVTCVVVDVSHEDPEVQFNWYVDGVEVHNAKTKPREEQFNSTFRVVSVLTVVHQDWLNGKEYKCKVSNKGLPAPIEKTISKTKGQPREPQVYTLPPSREEMTKNQVSLTCLVKGFYPSDISVEWESNGQPENNYKTTPPMLDSDGSFFLYSKLTVDKSRWQQGNVFSCSVMHEALHNHYTQKSLSLSPGK

SEQ ID NO: 3 - protein, 377 aa, Homo sapiens
ASTKGPSVFPLAPCSRSTSGGTAALGCLVKDYFPEPVTVSWNSGALTSGVHTFPAVLQSSGLYSLSSVVTVPSSSLGTQTYTCNVNHKPSNTKVDKRVELKTPLGDTTHTCPRCPEPKSCDTPPPCPRCPEPKSCDTPPPCPRCPEPKSCDTPPPCPRCPAPELLGGPSVFLFPPKPKDTLMISRTPEVTCVVVDVSHEDPEVQFKWYVDGVEVHNAKTKPREEQYNSTFRVVSVLTVLHQDWLNGKEYKCKVSNKALPAPIEKTISKTKGQPREPQVYTLPPSREEMTKNQVSLTCLVKGFYPSDIAVEWESSGQPENNYNTTPPMLDSDGSFFLYSKLTVDKSRWQQGNIFSCSVMHEALHNRFTQKSLSLSPGK

SEQ ID NO: 4 - protein, 327 aa, Homo sapiens
ASTKGPSVFPLAPCSRSTSESTAALGCLVKDYFPEPVTVSWNSGALTSGVHTFPAVLQSSGLYSLSSVVTVPSSSLGTKTYTCNVDHKPSNTKVDKRVESKYGPPCPSCPAPEFLGGPSVFLFPPKPKDTLMISRTPEVTCVVVDVSQEDPEVQFNWYVDGVEVHNAKTKPREEQFNSTYRVVSVLTVLHQDWLNGKEYKCKVSNKGLPSSIEKTISKAKGQPREPQVYTLPPSQEEMTKNQVSLTCLVKGFYPSDIAVEWESNGQPENNYKTTPPVLDSDGSFFLYSRLTVDKSRWQEGNVFSCSVMHEALHNHYTQKSLSLSLGK

SEQ ID NO: 5 - protein, 324 aa, Mus musculus
AKTTPPSVYPLAPGSAAQTNSMVTLGCLVKGYFPEPVTVTWNSGSLSSGVHTFPAVLQSDLYTLSSSVTVPSSPRPSETVTCNVAHPASSTKVDKKIVPRDCGCKPCICTVPEVSSVFIFPPKPKDVLTITLTPKVTCVVVDISKDDPEVQFSWFVDDVEVHTAQTQPREEQFNSTFRSVSELPIMHQDWLNGKEFKCRVNSAAFPAPIEKTISKTKGRPKAPQVYTIPPPKEQMAKDKVSLTCMITDFFPEDITVEWQWNGQPAENYKNTQPIMNTNGSYFVYSKLNVQKSNWEAGNTFTCSVLHEGLHNHHTEKSLSHSPGK

SEQ ID NO: 6 - protein, 330 aa, Mus musculus
AKTTAPSVYPLAPVCGDTTGSSVTLGCLVKGYFPEPVTLTWNSGSLSSGVHTFPAVLQSDLYTLSSSVTVTSSTWPSQSITCNVAHPASSTKVDKKIEPRGPTIKPCPPCKCPAPNLLGGPSVFIFPPKIKDVLMISLSPIVTCVVVDVSEDDPDVQISWFVNNVEVHTAQTQTHREDYNSTLRVVSALPIQHQDWMSGKEFKCKVNNKDLPAPIERTISKPKGSVRAPQVYVLPPPEEEMTKKQVTLTCMVTDFMPEDIYVEWTNNGKTELNYKNTEPVLDSDGSYFMYSKLRVEKKNWVERNSYSCSVVHEGLHNHHTTKSFSRTPGK

SEQ ID NO: 7 - protein, 335 aa, Mus musculus
KTTPPSVYPLAPGCGDTTGSSVTLGCLVKGYFPESVTVTWNSGSLSSSVHTFPALLQSGLYTMSSSVTVPSSTWPSQTVTCSVAHPASSTTVDKKLEPSGPISTINPCPPCKECHKCPAPNLEGGPSVFIFPPNIKDVLMISLTPKVTCVVVDVSEDDPDVQISWFVNNVEVHTAQTQTHREDYNSTIRVVSTLPIQHQDWMSGKEFKCKVNNKDLPSPIERTISKIKGLVRAPQVYILPPPAEQLSRKDVSLTCLVVGFNPGDISVEWTSNGHTEENYKDTAPVLDSDGSYFIYSKLNMKTSKWEKTDSFSCNVRHEGLKNYYLKKTISRSPGK

SEQ ID NO: 8 - protein, 329 aa, Mus musculus
TTTAPSVYPLVPGCSDTSGSSVTLGCLVKGYFPEPVTVKWNYGALSSGVRTVSSVLQSGFYSLSSLVTVPSSTWPSQTVICNVAHPASKTELIKRIEPRIPKPSTPPGSSCPPGNILGGPSVFIFPPKPKDALMISLTPKVTCVVVDVSEDDPDVHVSWFVDNKEVHTAWTQPREAQYNSTFRVVSALPIQHQDWMRGKEFKCKVNNKALPAPIERTISKPKGRAQTPQVYTIPPPREQMSKKKVSLTCLVTNFFSEAISVEWERNGELEQDYKNTPPILDSDGTYFLYSKLTVDTDSWLQGEIFTCSVVHEALHNHHTQKNLSRSPGK

SEQ ID NO: 9 - protein, 326 aa, Rattus norvegicus
AETTAPSVYPLAPGTALKSNSMVTLGCLVKGYFPEPVTVTWNSGALSSGVHTFPAVLQSGLYTLTSSVTVPSSTWPSQTVTCNVAHPASSTKVDKKIVPRNCGGDCKPCICTGSEVSSVFIFPPKPKDVLTITLTPKVTCVVVDISQDDPEVHFSWFVDDVEVHTAQTRPPEEQFNSTFRSVSELPILHQDWLNGRTFRCKVTSAAFPSPIEKTISKPEGRTQVPHVYTMSPTKEEMTQNEVSITCMVKGFYPPDIYVEWQMNGQPQENYKNTPPTMDTDGSYFLYSKLNVKKEKWQQGNTFTCSVLHEGLHNHHTEKSLSHSPGK

SEQ ID NO: 10 - protein, 322 aa, Rattus norvegicus
AETTAPSVYPLAPGTALKSNSMVTLGCLVKGYFPEPVTVTWNSGALSSGVHTFPAVLQSGLYTLTSSVTVPSSTWSSQAVTCNVAHPASSTKVDKKIVPRECNPCGCTGSEVSSVFIFPPKTKDVLTITLTPKVTCVVVDISQNDPEVRFSWFIDDVEVHTAQTHAPEKQSNSTLRSVSELPIVHRDWLNGKTFKCKVNSGAFPAPIEKSISKPEGTPRGPQVYTMAPPKEEMTQSQVSITCMVKGFYPPDIYTEWKMNGQPQENYKNTPPTMDTDGSYFLYSKLNVKKETWQQGNTFTCSVLHEGLHNHHTEKSLSHSPGK

SEQ ID NO: 11 - protein, 333 aa, Rattus norvegicus
AQTTAPSVYPLAPGCGDTTSSTVTLGCLVKGYFPEPVTVTWNSGALSSDVHTFPAVLQSGLYTLTSSVTSSTWPSQTVTCNVAHPASSTKVDKKVERRNGGIGHKCPTCPTCHKCPVPELLGGPSVFIFPPKPKDILLISQNAKVTCVVVDVSEEEPDVQFSWFVNNVEVHTAQTQPREEQYNSTFRVVSALPIQHQDWMSGKEFKCKVNNKALPSPIEKTISKPKGLVRKPQVYVMGPPTEQLTEQTVSLTCLTSGFLPNDIGVEWTSNGHIEKNYKNTEPVMDSDGSFFMYSKLNVERSRWDSRAPFVCSVVHEGLHNHHVEKSISRPPGK

SEQ ID NO: 12 - protein, 329 aa, Rattus norvegicus
ARTTAPSVYPLVPGCSGTSGSLVTLGCLVKGYFPEPVTVKWNSGALSSGVHTFPAVLQSGLYTLSSSVTVPSSTWSSQTVTCSVAHPATKSNLIKRIEPRRPKPRPPTDICSCDDNLGRPSVFIFPPKPKDILMITLTPKVTCVVVDVSEEEPDVQFSWFVDNVRVFTAQTQPHEEQLNGTFRVVSTLHIQHQDWMSGKEFKCKVNNKDLPSPIEKTISKPRGKARTPQVYTIPPPREQMSKNKVSLTCMVTSFYPASISVEWERNGELEQDYKNTLPVLDSDESYFLYSKLSVDTDSWMRGDIYTCSVVHEALHNHHTQKNLSRSPGK

SEQ ID NO: 13 - protein, 323 aa, Oryctolagus cuniculus
GQPKAPSVFPLAPCCGDTPSSTVTLGCLVKGYLPEPVTVTWNSGTLTNGVRTFPSVRQSSGLYSLSSVVSVTSSSQPVTCNVAHPATNTKVDKTVAPSTCSKPTCPPPELLGGPSVFIFPPKPKDTLMISRTPEVTCVVVDVSQDDPEVQFTWYINNEQVRTARPPLREQQFNSTIRVVSTLPITHQDWLRGKEFKCKVHNKALPAPIEKTISKARGQPLEPKVYTMGPPREELSSRSVSLTCMINGFYPSDISVEWEKNGKAEDNYKTTPAVLDSDGSYFLYNKLSVPTSEWQRGDVFTCSVMHEALHNHYTQKSISRSPGK

SEQ ID NO: 14 - protein, 330 aa, Artificial Sequence
  N180D
ASTKGPSVFPLAPSSKSTSGGTAALGCLVKDYFPEPVTVSWNSGALTSGVHTFPAVLQSSGLYSLSSVVTVPSSSLGTQTYICNVNHKPSNTKVDKKVEPKSCDKTHTCPPCPAPELLGGPSVFLFPPKPKDTLMISRTPEVTCVVVDVSHEDPEVKFNWYVDGVEVHNAKTKPREEQYDSTYRVVSVLTVLHQDWLNGKEYKCKVSNKALPAPIEKTISKAKGQPREPQVYTLPPSRDELTKNQVSLTCLVKGFYPSDIAVEWESNGQPENNYKTTPPVLDSDGSFFLYSKLTVDKSRWQQGNVFSCSVMHEALHNHYTQKSLSLSPGK

SEQ ID NO: 15 - protein, 326 aa, Artificial Sequence
  N176D
ASTKGPSVFPLAPCSRSTSESTAALGCLVKDYFPEPVTVSWNSGALTSGVHTFPAVLQSSGLYSLSSVVTVPSSNFGTQTYTCNVDHKPSNTKVDKTVERKCCVECPPCPAPPVAGPSVFLFPPKPKDTLMISRTPEVTCVVVDVSHEDPEVQFNWYVDGVEVHNAKTKPREEQFDSTFRVVSVLTVVHQDWLNGKEYKCKVSNKGLPAPIEKTISKTKGQPREPQVYTLPPSREEMTKNQVSLTCLVKGFYPSDISVEWESNGQPENNYKTTPPMLDSDGSFFLYSKLTVDKSRWQQGNVFSCSVMHEALHNHYTQKSLSLSPGK

SEQ ID NO: 16 - protein, 377 aa, Artificial Sequence
  N227D
ASTKGPSVFPLAPCSRSTSGGTAALGCLVKDYFPEPVTVSWNSGALTSGVHTFPAVLQSSGLYSLSSVVTVPSSSLGTQTYTCNVNHKPSNTKVDKRVELKTPLGDTTHTCPRCPEPKSCDTPPPCPRCPEPKSCDTPPPCPRCPEPKSCDTPPPCPRCPAPELLGGPSVFLFPPKPKDTLMISRTPEVTCVVVDVSHEDPEVQFKWYVDGVEVHNAKTKPREEQYDSTFRVVSVLTVLHQDWLNGKEYKCKVSNKALPAPIEKTISKTKGQPREPQVYTLPPSREEMTKNQVSLTCLVKGFYPSDIAVEWESSGQPENNYNTTPPMLDSDGSFFLYSKLTVDKSRWQQGNIFSCSVMHEALHNRFTQKSLSLSPGK

SEQ ID NO: 17 - protein, 327 aa, Artificial Sequence
  N177D
ASTKGPSVFPLAPCSRSTSESTAALGCLVKDYFPEPVTVSWNSGALTSGVHTFPAVLQSSGLYSLSSVVTVPSSSLGTKTYTCNVDHKPSNTKVDKRVESKYGPPCPSCPAPEFLGGPSVFLFPPKPKDTLMISRTPEVTCVVVDVSQEDPEVQFNWYVDGVEVHNAKTKPREEQFDSTYRVVSVLTVLHQDWLNGKEYKCKVSNKGLPSSIEKTISKAKGQPREPQVYTLPPSQEEMTKNQVSLTCLVKGFYPSDIAVEWESNGQPENNYKTTPPVLDSDGSFFLYSRLTVDKSRWQEGNVFSCSVMHEALHNHYTQKSLSLSLGK

SEQ ID NO: 18 - protein, 324 aa, Artificial Sequence
  N174D
AKTTPPSVYPLAPGSAAQTNSMVTLGCLVKGYFPEPVTVTWNSGSLSSGVHTFPAVLQSDLYTLSSSVTVPSSPRPSETVTCNVAHPASSTKVDKKIVPRDCGCKPCICTVPEVSSVFIFPPKPKDVLTITLTPKVTCVVVDISKDDPEVQFSWFVDDVEVHTAQTQPREEQFDSTFRSVSELPIMHQDWLNGKEFKCRVNSAAFPAPIEKTISKTKGRPKAPQVYTIPPPKEQMAKDKVSLTCMITDFFPEDITVEWQWNGQPAENYKNTQPIMNTNGSYFVYSKLNVQKSNWEAGNTFTCSVLHEGLHNHHTEKSLSHSPGK

SEQ ID NO: 19 - protein, 330 aa, Artificial Sequence
  N180D
AKTTAPSVYPLAPVCGDTTGSSVTLGCLVKGYFPEPVTLTWNSGSLSSGVHTFPAVLQSDLYTLSSSVTVTSSTWPSQSITCNVAHPASSTKVDKKIEPRGPTIKPCPPCKCPAPNLLGGPSVFIFPPKIKDVLMISLSPIVTCVVVDVSEDDPDVQISWFVNNVEVHTAQTQTHREDYDSTLRVVSALPIQHQDWMSGKEFKCKVNNKDLPAPIERTISKPKGSVRAPQVYVLPPPEEEMTKKQVTLTCMVTDFMPEDIYVEWTNNGKTELNYKNTEPVLDSDGSYFMYSKLRVEKKNWVERNSYSCSVVHEGLHNHHTTKSFSRTPGK

SEQ ID NO: 20 - protein, 335 aa, Artificial Sequence
  N185D
KTTPPSVYPLAPGCGDTTGSSVTLGCLVKGYFPESVTVTWNSGSLSSSVHTFPALLQSGLYTMSSSVTVPSSTWPSQTVTCSVAHPASSTTVDKKLEPSGPISTINPCPPCKECHKCPAPNLEGGPSVFIFPPNIKDVLMISLTPKVTCVVVDVSEDDPDVQISWFVNNVEVHTAQTQTHREDYDSTIRVVSTLPIQHQDWMSGKEFKCKVNNKDLPSPIERTISKIKGLVRAPQVYILPPPAEQLSRKDVSLTCLVVGFNPGDISVEWTSNGHTEENYKDTAPVLDSDGSYFIYSKLNMKTSKWEKTDSFSCNVRHEGLKNYYLKKTISRSPGK

SEQ ID NO: 21 - protein, 329 aa, Artificial Sequence
  N179D
TTTAPSVYPLVPGCSDTSGSSVTLGCLVKGYFPEPVTVKWNYGALSSGVRTVSSVLQSGFYSLSSLVTVPSSTWPSQTVICNVAHPASKTELIKRIEPRIPKPSTPPGSSCPPGNILGGPSVFIFPPKPKDALMISLTPKVTCVVVDVSEDDPDVHVSWFVDNKEVHTAWTQPREAQYDSTFRVVSALPIQHQDWMRGKEFKCKVNNKALPAPIERTISKPKGRAQTPQVYTIPPPREQMSKKKVSLTCLVTNFFSEAISVEWERNGELEQDYKNTPPILDSDGTYFLYSKLTVDTDSWLQGEIFTCSVVHEALHNHHTQKNLSRSPGK

SEQ ID NO: 22 - protein, 326 aa, Artificial Sequence
  N176D
AETTAPSVYPLAPGTALKSNSMVTLGCLVKGYFPEPVTVTWNSGALSSGVHTFPAVLQSGLYTLTSSVTVPSSTWPSQTVTCNVAHPASSTKVDKKIVPRNCGGDCKPCICTGSEVSSVFIFPPKPKDVLTITLTPKVTCVVVDISQDDPEVHFSWFVDDVEVHTAQTRPPEEQFDSTFRSVSELPILHQDWLNGRTFRCKVTSAAFPSPIEKTISKPEGRTQVPHVYTMSPTKEEMTQNEVSITCMVKGFYPPDIYVEWQMNGQPQENYKNTPPTMDTDGSYFLYSKLNVKKEKWQQGNTFTCSVLHEGLHNHHTEKSLSHSPGK

SEQ ID NO: 23 - protein, 322 aa, Artificial Sequence
  N172D
AETTAPSVYPLAPGTALKSNSMVTLGCLVKGYFPEPVTVTWNSGALSSGVHTFPAVLQSGLYTLTSSVTVPSSTWSSQAVTCNVAHPASSTKVDKKIVPRECNPCGCTGSEVSSVFIFPPKTKDVLTITLTPKVTCVVVDISQNDPEVRFSWFIDDVEVHTAQTHAPEKQSDSTLRSVSELPIVHRDWLNGKTFKCKVNSGAFPAPIEKSISKPEGTPRGPQVYTMAPPKEEMTQSQVSITCMVKGFYPPDIYTEWKMNGQPQENYKNTPPTMDTDGSYFLYSKLNVKKETWQQGNTFTCSVLHEGLHNHHTEKSLSHSPGK

SEQ ID NO: 24 - protein, 333 aa, Artificial Sequence
  N183D
AQTTAPSVYPLAPGCGDTTSSTVTLGCLVKGYFPEPVTVTWNSGALSSDVHTFPAVLQSGLYTLTSSVTSSTWPSQTVTCNVAHPASSTKVDKKVERRNGGIGHKCPTCPTCHKCPVPELLGGPSVFIFPPKPKDILLISQNAKVTCVVVDVSEEEPDVQFSWFVNNVEVHTAQTQPREEQYDSTFRVVSALPIQHQDWMSGKEFKCKVNNKALPSPIEKTISKPKGLVRKPQVYVMGPPTEQLTEQTVSLTCLTSGFLPNDIGVEWTSNGHIEKNYKNTEPVMDSDGSFFMYSKLNVERSRWDSRAPFVCSVVHEGLHNHHVEKSISRPPGK

SEQ ID NO: 25 - protein, 329 aa, Artificial Sequence
  N179D
ARTTAPSVYPLVPGCSGTSGSLVTLGCLVKGYFPEPVTVKWNSGALSSGVHTFPAVLQSGLYTLSSSVTVPSSTWSSQTVTCSVAHPATKSNLIKRIEPRRPKPRPPTDICSCDDNLGRPSVFIFPPKPKDILMITLTPKVTCVVVDVSEEEPDVQFSWFVDNVRVFTAQTQPHEEQLDGTFRVVSTLHIQHQDWMSGKEFKCKVNNKDLPSPIEKTISKPRGKARTPQVYTIPPPREQMSKNKVSLTCMVTSFYPASISVEWERNGELEQDYKNTLPVLDSDESYFLYSKLSVDTDSWMRGDIYTCSVVHEALHNHHTQKNLSRSPGK

SEQ ID NO: 26 - protein, 323 aa, Artificial Sequence
  N173D
GQPKAPSVFPLAPCCGDTPSSTVTLGCLVKGYLPEPVTVTWNSGTLTNGVRTFPSVRQSSGLYSLSSVVSVTSSSQPVTCNVAHPATNTKVDKTVAPSTCSKPTCPPPELLGGPSVFIFPPKPKDTLMISRTPEVTCVVVDVSQDDPEVQFTWYINNEQVRTARPPLREQQFDSTIRVVSTLPITHQDWLRGKEFKCKVHNKALPAPIEKTISKARGQPLEPKVYTMGPPREELSSRSVSLTCMINGFYPSDISVEWEKNGKAEDNYKTTPAVLDSDGSYFLYNKLSVPTSEWQRGDVFTCSVMHEALHNHYTQKSISRSPGK

SEQ ID NO: 27 - protein, 330 aa, Artificial Sequence
  N180Q
ASTKGPSVFPLAPSSKSTSGGTAALGCLVKDYFPEPVTVSWNSGALTSGVHTFPAVLQSSGLYSLSSVVTVPSSSLGTQTYICNVNHKPSNTKVDKKVEPKSCDKTHTCPPCPAPELLGGPSVFLFPPKPKDTLMISRTPEVTCVVVDVSHEDPEVKFNWYVDGVEVHNAKTKPREEQYQSTYRVVSVLTVLHQDWLNGKEYKCKVSNKALPAPIEKTISKAKGQPREPQVYTLPPSRDELTKNQVSLTCLVKGFYPSDIAVEWESNGQPENNYKTTPPVLDSDGSFFLYSKLTVDKSRWQQGNVFSCSVMHEALHNHYTQKSLSLSPGK

SEQ ID NO: 28 - protein, 326 aa, Artificial Sequence
  N176Q
ASTKGPSVFPLAPCSRSTSESTAALGCLVKDYFPEPVTVSWNSGALTSGVHTFPAVLQSSGLYSLSSVVTVPSSNFGTQTYTCNVDHKPSNTKVDKTVERKCCVECPPCPAPPVAGPSVFLFPPKPKDTLMISRTPEVTCVVVDVSHEDPEVQFNWYVDGVEVHNAKTKPREEQFQSTFRVVSVLTVVHQDWLNGKEYKCKVSNKGLPAPIEKTISKTKGQPREPQVYTLPPSREEMTKNQVSLTCLVKGFYPSDISVEWESNGQPENNYKTTPPMLDSDGSFFLYSKLTVDKSRWQQGNVFSCSVMHEALHNHYTQKSLSLSPGK

SEQ ID NO: 29 - protein, 377 aa, Artificial Sequence
  N227Q
ASTKGPSVFPLAPCSRSTSGGTAALGCLVKDYFPEPVTVSWNSGALTSGVHTFPAVLQSSGLYSLSSVVTVPSSSLGTQTYTCNVNHKPSNTKVDKRVELKTPLGDTTHTCPRCPEPKSCDTPPPCPRCPEPKSCDTPPPCPRCPEPKSCDTPPPCPRCPAPELLGGPSVFLFPPKPKDTLMISRTPEVTCVVVDVSHEDPEVQFKWYVDGVEVHNAKTKPREEQYQSTFRVVSVLTVLHQDWLNGKEYKCKVSNKALPAPIEKTISKTKGQPREPQVYTLPPSREEMTKNQVSLTCLVKGFYPSDIAVEWESSGQPENNYNTTPPMLDSDGSFFLYSKLTVDKSRWQQGNIFSCSVMHEALHNRFTQKSLSLSPGK

SEQ ID NO: 30 - protein, 327 aa, Artificial Sequence
  N177Q
ASTKGPSVFPLAPCSRSTSESTAALGCLVKDYFPEPVTVSWNSGALTSGVHTFPAVLQSSGLYSLSSVVTVPSSSLGTKTYTCNVDHKPSNTKVDKRVESKYGPPCPSCPAPEFLGGPSVFLFPPKPKDTLMISRTPEVTCVVVDVSQEDPEVQFNWYVDGVEVHNAKTKPREEQFQSTYRVVSVLTVLHQDWLNGKEYKCKVSNKGLPSSIEKTISKAKGQPREPQVYTLPPSQEEMTKNQVSLTCLVKGFYPSDIAVEWESNGQPENNYKTTPPVLDSDGSFFLYSRLTVDKSRWQEGNVFSCSVMHEALHNHYTQKSLSLSLGK

SEQ ID NO: 31 - protein, 324 aa, Artificial Sequence
  N174Q
AKTTPPSVYPLAPGSAAQTNSMVTLGCLVKGYFPEPVTVTWNSGSLSSGVHTFPAVLQSDLYTLSSSVTVPSSPRPSETVTCNVAHPASSTKVDKKIVPRDCGCKPCICTVPEVSSVFIFPPKPKDVLTITLTPKVTCVVVDISKDDPEVQFSWFVDDVEVHTAQTQPREEQFQSTFRSVSELPIMHQDWLNGKEFKCRVNSAAFPAPIEKTISKTKGRPKAPQVYTIPPPKEQMAKDKVSLTCMITDFFPEDITVEWQWNGQPAENYKNTQPIMNTNGSYFVYSKLNVQKSNWEAGNTFTCSVLHEGLHNHHTEKSLSHSPGK

SEQ ID NO: 32 - protein, 330 aa, Artificial Sequence
  N180Q
AKTTAPSVYPLAPVCGDTTGSSVTLGCLVKGYFPEPVTLTWNSGSLSSGVHTFPAVLQSDLYTLSSSVTVTSSTWPSQSITCNVAHPASSTKVDKKIEPRGPTIKPCPPCKCPAPNLLGGPSVFIFPPKIKDVLMISLSPIVTCVVVDVSEDDPDVQISWFVNNVEVHTAQTQTHREDYQSTLRVVSALPIQHQDWMSGKEFKCKVNNKDLPAPIERTISKPKGSVRAPQVYVLPPPEEEMTKKQVTLTCMVTDFMPEDIYVEWTNNGKTELNYKNTEPVLDSDGSYFMYSKLRVEKKNWVERNSYSCSVVHEGLHNHHTTKSFSRTPGK

SEQ ID NO: 33 - protein, 335 aa, Artificial Sequence
  N185Q
KTTPPSVYPLAPGCGDTTGSSVTLGCLVKGYFPESVTVTWNSGSLSSSVHTFPALLQSGLYTMSSSVTVPSSTWPSQTVTCSVAHPASSTTVDKKLEPSGPISTINPCPPCKECHKCPAPNLEGGPSVFIFPPNIKDVLMISLTPKVTCVVVDVSEDDPDVQISWFVNNVEVHTAQTQTHREDYQSTIRVVSTLPIQHQDWMSGKEFKCKVNNKDLPSPIERTISKIKGLVRAPQVYILPPPAEQLSRKDVSLTCLVVGFNPGDISVEWTSNGHTEENYKDTAPVLDSDGSYFIYSKLNMKTSKWEKTDSFSCNVRHEGLKNYYLKKTISRSPGK

SEQ ID NO: 34 - protein, 329 aa, Artificial Sequence
  N179Q
TTTAPSVYPLVPGCSDTSGSSVTLGCLVKGYFPEPVTVKWNYGALSSGVRTVSSVLQSGFYSLSSLVTVPSSTWPSQTVICNVAHPASKTELIKRIEPRIPKPSTPPGSSCPPGNILGGPSVFIFPPKPKDALMISLTPKVTCVVVDVSEDDPDVHVSWFVDNKEVHTAWTQPREAQYQSTFRVVSALPIQHQDWMRGKEFKCKVNNKALPAPIERTISKPKGRAQTPQVYTIPPPREQMSKKKVSLTCLVTNFFSEAISVEWERNGELEQDYKNTPPILDSDGTYFLYSKLTVDTDSWLQGEIFTCSVVHEALHNHHTQKNLSRSPGK

SEQ ID NO: 35 - protein, 326 aa, Artificial Sequence
  N176Q
AETTAPSVYPLAPGTALKSNSMVTLGCLVKGYFPEPVTVTWNSGALSSGVHTFPAVLQSGLYTLTSSVTVPSSTWPSQTVTCNVAHPASSTKVDKKIVPRNCGGDCKPCICTGSEVSSVFIFPPKPKDVLTITLTPKVTCVVVDISQDDPEVHFSWFVDDVEVHTAQTRPPEEQFQSTFRSVSELPILHQDWLNGRTFRCKVTSAAFPSPIEKTISKPEGRTQVPHVYTMSPTKEEMTQNEVSITCMVKGFYPPDIYVEWQMNGQPQENYKNTPPTMDTDGSYFLYSKLNVKKEKWQQGNTFTCSVLHEGLHNHHTEKSLSHSPGK

SEQ ID NO: 36 - protein, 322 aa, Artificial Sequence
  N172Q
AETTAPSVYPLAPGTALKSNSMVTLGCLVKGYFPEPVTVTWNSGALSSGVHTFPAVLQSGLYTLTSSVTVPSSTWSSQAVTCNVAHPASSTKVDKKIVPRECNPCGCTGSEVSSVFIFPPKTKDVLTITLTPKVTCVVVDISQNDPEVRFSWFIDDVEVHTAQTHAPEKQSQSTLRSVSELPIVHRDWLNGKTFKCKVNSGAFPAPIEKSISKPEGTPRGPQVYTMAPPKEEMTQSQVSITCMVKGFYPPDIYTEWKMNGQPQENYKNTPPTMDTDGSYFLYSKLNVKKETWQQGNTFTCSVLHEGLHNHHTEKSLSHSPGK

SEQ ID NO: 37 - protein, 333 aa, Artificial Sequence
  N183Q
AQTTAPSVYPLAPGCGDTTSSTVTLGCLVKGYFPEPVTVTWNSGALSSDVHTFPAVLQSGLYTLTSSVTSSTWPSQTVTCNVAHPASSTKVDKKVERRNGGIGHKCPTCPTCHKCPVPELLGGPSVFIFPPKPKDILLISQNAKVTCVVVDVSEEEPDVQFSWFVNNVEVHTAQTQPREEQYQSTFRVVSALPIQHQDWMSGKEFKCKVNNKALPSPIEKTISKPKGLVRKPQVYVMGPPTEQLTEQTVSLTCLTSGFLPNDIGVEWTSNGHIEKNYKNTEPVMDSDGSFFMYSKLNVERSRWDSRAPFVCSVVHEGLHNHHVEKSISRPPGK

SEQ ID NO: 38 - protein, 329 aa, Artificial Sequence
  N179Q
ARTTAPSVYPLVPGCSGTSGSLVTLGCLVKGYFPEPVTVKWNSGALSSGVHTFPAVLQSGLYTLSSSVTVPSSTWSSQTVTCSVAHPATKSNLIKRIEPRRPKPRPPTDICSCDDNLGRPSVFIFPPKPKDILMITLTPKVTCVVVDVSEEEPDVQFSWFVDNVRVFTAQTQPHEEQLQGTFRVVSTLHIQHQDWMSGKEFKCKVNNKDLPSPIEKTISKPRGKARTPQVYTIPPPREQMSKNKVSLTCMVTSFYPASISVEWERNGELEQDYKNTLPVLDSDESYFLYSKLSVDTDSWMRGDIYTCSVVHEALHNHHTQKNLSRSPGK

SEQ ID NO: 39 - protein, 323 aa, Artificial Sequence
  N173Q
GQPKAPSVFPLAPCCGDTPSSTVTLGCLVKGYLPEPVTVTWNSGTLTNGVRTFPSVRQSSGLYSLSSVVSVTSSSQPVTCNVAHPATNTKVDKTVAPSTCSKPTCPPPELLGGPSVFIFPPKPKDTLMISRTPEVTCVVVDVSQDDPEVQFTWYINNEQVRTARPPLREQQFQSTIRVVSTLPITHQDWLRGKEFKCKVHNKALPAPIEKTISKARGQPLEPKVYTMGPPREELSSRSVSLTCMINGFYPSDISVEWEKNGKAEDNYKTTPAVLDSDGSYFLYNKLSVPTSEWQRGDVFTCSVMHEALHNHYTQKSISRSPGK

SEQ ID NO: 40 - protein, 330 aa, Artificial Sequence
  T182A
ASTKGPSVFPLAPSSKSTSGGTAALGCLVKDYFPEPVTVSWNSGALTSGVHTFPAVLQSSGLYSLSSVVTVPSSSLGTQTYICNVNHKPSNTKVDKKVEPKSCDKTHTCPPCPAPELLGGPSVFLFPPKPKDTLMISRTPEVTCVVVDVSHEDPEVKFNWYVDGVEVHNAKTKPREEQYNSAYRVVSVLTVLHQDWLNGKEYKCKVSNKALPAPIEKTISKAKGQPREPQVYTLPPSRDELTKNQVSLTCLVKGFYPSDIAVEWESNGQPENNYKTTPPVLDSDGSFFLYSKLTVDKSRWQQGNVFSCSVMHEALHNHYTQKSLSLSPGK

SEQ ID NO: 41 - protein, 326 aa, Artificial Sequence
  T178A
ASTKGPSVFPLAPCSRSTSESTAALGCLVKDYFPEPVTVSWNSGALTSGVHTFPAVLQSSGLYSLSSVVTVPSSNFGTQTYTCNVDHKPSNTKVDKTVERKCCVECPPCPAPPVAGPSVFLFPPKPKDTLMISRTPEVTCVVVDVSHEDPEVQFNWYVDGVEVHNAKTKPREEQFNSAFRVVSVLTVVHQDWLNGKEYKCKVSNKGLPAPIEKTISKTKGQPREPQVYTLPPSREEMTKNQVSLTCLVKGFYPSDISVEWESNGQPENNYKTTPPMLDSDGSFFLYSKLTVDKSRWQQGNVFSCSVMHEALHNHYTQKSLSLSPGK

SEQ ID NO: 42 - protein, 377 aa, Artificial Sequence
  T229A
ASTKGPSVFPLAPCSRSTSGGTAALGCLVKDYFPEPVTVSWNSGALTSGVHTFPAVLQSSGLYSLSSVVTVPSSSLGTQTYTCNVNHKPSNTKVDKRVELKTPLGDTTHTCPRCPEPKSCDTPPPCPRCPEPKSCDTPPPCPRCPEPKSCDTPPPCPRCPAPELLGGPSVFLFPPKPKDTLMISRTPEVTCVVVDVSHEDPEVQFKWYVDGVEVHNAKTKPREEQYNSAFRVVSVLTVLHQDWLNGKEYKCKVSNKALPAPIEKTISKTKGQPREPQVYTLPPSREEMTKNQVSLTCLVKGFYPSDIAVEWESSGQPENNYNTTPPMLDSDGSFFLYSKLTVDKSRWQQGNIFSCSVMHEALHNRFTQKSLSLSPGK

SEQ ID NO: 43 - protein, 327 aa, Artificial Sequence
  T179A
ASTKGPSVFPLAPCSRSTSESTAALGCLVKDYFPEPVTVSWNSGALTSGVHTFPAVLQSSGLYSLSSVVTVPSSSLGTKTYTCNVDHKPSNTKVDKRVESKYGPPCPSCPAPEFLGGPSVFLFPPKPKDTLMISRTPEVTCVVVDVSQEDPEVQFNWYVDGVEVHNAKTKPREEQFNSAYRVVSVLTVLHQDWLNGKEYKCKVSNKGLPSSIEKTISKAKGQPREPQVYTLPPSQEEMTKNQVSLTCLVKGFYPSDIAVEWESNGQPENNYKTTPPVLDSDGSFFLYSRLTVDKSRWQEGNVFSCSVMHEALHNHYTQKSLSLSLGK

SEQ ID NO: 44 - protein, 324 aa, Artificial Sequence
  T176A
AKTTPPSVYPLAPGSAAQTNSMVTLGCLVKGYFPEPVTVTWNSGSLSSGVHTFPAVLQSDLYTLSSSVTVPSSPRPSETVTCNVAHPASSTKVDKKIVPRDCGCKPCICTVPEVSSVFIFPPKPKDVLTITLTPKVTCVVVDISKDDPEVQFSWFVDDVEVHTAQTQPREEQFNSAFRSVSELPIMHQDWLNGKEFKCRVNSAAFPAPIEKTISKTKGRPKAPQVYTIPPPKEQMAKDKVSLTCMITDFFPEDITVEWQWNGQPAENYKNTQPIMNTNGSYFVYSKLNVQKSNWEAGNTFTCSVLHEGLHNHHTEKSLSHSPGK

SEQ ID NO: 45 - protein, 330 aa, Artificial Sequence
  T182A
AKTTAPSVYPLAPVCGDTTGSSVTLGCLVKGYFPEPVTLTWNSGSLSSGVHTFPAVLQSDLYTLSSSVTVTSSTWPSQSITCNVAHPASSTKVDKKIEPRGPTIKPCPPCKCPAPNLLGGPSVFIFPPKIKDVLMISLSPIVTCVVVDVSEDDPDVQISWFVNNVEVHTAQTQTHREDYNSALRVVSALPIQHQDWMSGKEFKCKVNNKDLPAPIERTISKPKGSVRAPQVYVLPPPEEEMTKKQVTLTCMVTDFMPEDIYVEWTNNGKTELNYKNTEPVLDSDGSYFMYSKLRVEKKNWVERNSYSCSVVHEGLHNHHTTKSFSRTPGK

SEQ ID NO: 46 - protein, 335 aa, Artificial Sequence
  T187A
KTTPPSVYPLAPGCGDTTGSSVTLGCLVKGYFPESVTVTWNSGSLSSSVHTFPALLQSGLYTMSSSVTVPSSTWPSQTVTCSVAHPASSTTVDKKLEPSGPISTINPCPPCKECHKCPAPNLEGGPSVFIFPPNIKDVLMISLTPKVTCVVVDVSEDDPDVQISWFVNNVEVHTAQTQTHREDYNSAIRVVSTLPIQHQDWMSGKEFKCKVNNKDLPSPIERTISKIKGLVRAPQVYILPPPAEQLSRKDVSLTCLVVGFNPGDISVEWTSNGHTEENYKDTAPVLDSDGSYFIYSKLNMKTSKWEKTDSFSCNVRHEGLKNYYLKKTISRSPGK

SEQ ID NO: 47 - protein, 329 aa, Artificial Sequence
  T181A
TTTAPSVYPLVPGCSDTSGSSVTLGCLVKGYFPEPVTVKWNYGALSSGVRTVSSVLQSGFYSLSSLVTVPSSTWPSQTVICNVAHPASKTELIKRIEPRIPKPSTPPGSSCPPGNILGGPSVFIFPPKPKDALMISLTPKVTCVVVDVSEDDPDVHVSWFVDNKEVHTAWTQPREAQYNSAFRVVSALPIQHQDWMRGKEFKCKVNNKALPAPIERTISKPKGRAQTPQVYTIPPPREQMSKKKVSLTCLVTNFFSEAISVEWERNGELEQDYKNTPPILDSDGTYFLYSKLTVDTDSWLQGEIFTCSVVHEALHNHHTQKNLSRSPGK

SEQ ID NO: 48 - protein, 326 aa, Artificial Sequence
  T178A
AETTAPSVYPLAPGTALKSNSMVTLGCLVKGYFPEPVTVTWNSGALSSGVHTFPAVLQSGLYTLTSSVTVPSSTWPSQTVTCNVAHPASSTKVDKKIVPRNCGGDCKPCICTGSEVSSVFIFPPKPKDVLTITLTPKVTCVVVDISQDDPEVHFSWFVDDVEVHTAQTRPPEEQFNSAFRSVSELPILHQDWLNGRTFRCKVTSAAFPSPIEKTISKPEGRTQVPHVYTMSPTKEEMTQNEVSITCMVKGFYPPDIYVEWQMNGQPQENYKNTPPTMDTDGSYFLYSKLNVKKEKWQQGNTFTCSVLHEGLHNHHTEKSLSHSPGK

SEQ ID NO: 49 - protein, 322 aa, Artificial Sequence
  T174A
AETTAPSVYPLAPGTALKSNSMVTLGCLVKGYFPEPVTVTWNSGALSSGVHTFPAVLQSGLYTLTSSVTVPSSTWSSQAVTCNVAHPASSTKVDKKIVPRECNPCGCTGSEVSSVFIFPPKTKDVLTITLTPKVTCVVVDISQNDPEVRFSWFIDDVEVHTAQTHAPEKQSNSALRSVSELPIVHRDWLNGKTFKCKVNSGAFPAPIEKSISKPEGTPRGPQVYTMAPPKEEMTQSQVSITCMVKGFYPPDIYTEWKMNGQPQENYKNTPPTMDTDGSYFLYSKLNVKKETWQQGNTFTCSVLHEGLHNHHTEKSLSHSPGK

SEQ ID NO: 50 - protein, 333 aa, Artificial Sequence
  T185A
AQTTAPSVYPLAPGCGDTTSSTVTLGCLVKGYFPEPVTVTWNSGALSSDVHTFPAVLQSGLYTLTSSVTSSTWPSQTVTCNVAHPASSTKVDKKVERRNGGIGHKCPTCPTCHKCPVPELLGGPSVFIFPPKPKDILLISQNAKVTCVVVDVSEEEPDVQFSWFVNNVEVHTAQTQPREEQYNSAFRVVSALPIQHQDWMSGKEFKCKVNNKALPSPIEKTISKPKGLVRKPQVYVMGPPTEQLTEQTVSLTCLTSGFLPNDIGVEWTSNGHIEKNYKNTEPVMDSDGSFFMYSKLNVERSRWDSRAPFVCSVVHEGLHNHHVEKSISRPPGK

SEQ ID NO: 51 - protein, 329 aa, Artificial Sequence
  T181A
ARTTAPSVYPLVPGCSGTSGSLVTLGCLVKGYFPEPVTVKWNSGALSSGVHTFPAVLQSGLYTLSSSVTVPSSTWSSQTVTCSVAHPATKSNLIKRIEPRRPKPRPPTDICSCDDNLGRPSVFIFPPKPKDILMITLTPKVTCVVVDVSEEEPDVQFSWFVDNVRVFTAQTQPHEEQLNGAFRVVSTLHIQHQDWMSGKEFKCKVNNKDLPSPIEKTISKPRGKARTPQVYTIPPPREQMSKNKVSLTCMVTSFYPASISVEWERNGELEQDYKNTLPVLDSDESYFLYSKLSVDTDSWMRGDIYTCSVVHEALHNHHTQKNLSRSPGK

SEQ ID NO: 52 - protein, 323 aa, Artificial Sequence
  T175A
GQPKAPSVFPLAPCCGDTPSSTVTLGCLVKGYLPEPVTVTWNSGTLTNGVRTFPSVRQSSGLYSLSSVVSVTSSSQPVTCNVAHPATNTKVDKTVAPSTCSKPTCPPPELLGGPSVFIFPPKPKDTLMISRTPEVTCVVVDVSQDDPEVQFTWYINNEQVRTARPPLREQQFNSAIRVVSTLPITHQDWLRGKEFKCKVHNKALPAPIEKTISKARGQPLEPKVYTMGPPREELSSRSVSLTCMINGFYPSDISVEWEKNGKAEDNYKTTPAVLDSDGSYFLYNKLSVPTSEWQRGDVFTCSVMHEALHNHYTQKSISRSPGK